European Patent Application EP 4 458 837 A1, published November 6, 2024. Title: Peptide having activities of skin condition improvement and uses thereof. Applicant: CAREGEN CO., LTD. The sequence listing filed with the application follows.

SEQUENCE LISTING (13 sequences)

SEQ ID NO: 1 - protein, 5 aa, Artificial Sequence
  Peptide 1
DGFND

SEQ ID NO: 2 - DNA, 20 bp, Artificial Sequence
  Col1a1_F
caccctcaagagcctgagtc

SEQ ID NO: 3 - DNA, 20 bp, Artificial Sequence
  Col1a1_R
agacggctgagtagggaaca

SEQ ID NO: 4 - DNA, 20 bp, Artificial Sequence
  Fibronectin_F
ccaggaaccgagtacaccat

SEQ ID NO: 5 - DNA, 20 bp, Artificial Sequence
  Fibronectin_R
atacccaggttgggtgatga

SEQ ID NO: 6 - DNA, 20 bp, Artificial Sequence
  Elastin_F
gcaagacctggctttggact

SEQ ID NO: 7 - DNA, 21 bp, Artificial Sequence
  Elastin_R
gggagtttctggttagggctg

SEQ ID NO: 8 - DNA, 20 bp, Artificial Sequence
  GAPDH_F
ggagccaaaagggtcatcat

SEQ ID NO: 9 - DNA, 20 bp, Artificial Sequence
  GAPDH_R
gtgatggcatggactgtggt

SEQ ID NO: 10 - DNA, 20 bp, Artificial Sequence
  SIRT1_F
tcagtggctggaacagtgag

SEQ ID NO: 11 - DNA, 20 bp, Artificial Sequence
  SIRT1_R
tctggcatgtcccactatca

SEQ ID NO: 12 - DNA, 20 bp, Artificial Sequence
  AQP3_F
ccttcttgggtgctggaata

SEQ ID NO: 13 - DNA, 20 bp, Artificial Sequence
  AQP3_R
acacgataagggaggctgtg